European Patent Application EP 4 382 170 A2, published June 12, 2024. Title: Factor VIII-Fc chimeric and hybrid polypeptides, and methods of use thereof. Applicant: Bioverative Therapeutics Inc. Application EP. The sequence listing filed with the application follows.

SEQUENCE LISTING (12 sequences)

SEQ ID NO: 1 - DNA, 5052 bp, synthetic construct
  misc_feature 1..5052: note = B-Domain Deleted FVIIIFc Chain
  misc_feature 1..57: note = FVIII signal
  misc_feature 4372..5052: note = Fc region
  source 1..5052: mol_type = other DNA
atgcaaatagagctctccacctgcttctttctgtgccttttgcgattctgctttagtgccaccagaagatactacctgggtgcagtggaactgtcatgggactatatgcaaagtgatctcggtgagctgcctgtggacgcaagatttcctcctagagtgccaaaatcttttccattcaacacctcagtcgtgtacaaaaagactctgtttgtagaattcacggatcaccttttcaacatcgctaagccaaggccaccctggatgggtctgctaggtcctaccatccaggctgaggtttatgatacagtggtcattacacttaagaacatggcttcccatcctgtcagtcttcatgctgttggtgtatcctactggaaagcttctgagggagctgaatatgatgatcagaccagtcaaagggagaaagaagatgataaagtcttccctggtggaagccatacatatgtctggcaggtcctgaaagagaatggtccaatggcctctgacccactgtgccttacctactcatatctttctcatgtggacctggtaaaagacttgaattcaggcctcattggagccctactagtatgtagagaagggagtctggccaaggaaaagacacagaccttgcacaaatttatactactttttgctgtatttgatgaagggaaaagttggcactcagaaacaaagaactccttgatgcaggatagggatgctgcatctgctcgggcctggcctaaaatgcacacagtcaatggttatgtaaacaggtctctgccaggtctgattggatgccacaggaaatcagtctattggcatgtgattggaatgggcaccactcctgaagtgcactcaatattcctcgaaggtcacacatttcttgtgaggaaccatcgccaggcgtccttggaaatctcgccaataactttccttactgctcaaacactcttgatggaccttggacagtttctactgttttgtcatatctcttcccaccaacatgatggcatggaagcttatgtcaaagtagacagctgtccagaggaaccccaactacgaatgaaaaataatgaagaagcggaagactatgatgatgatcttactgattctgaaatggatgtggtcaggtttgatgatgacaactctccttcctttatccaaattcgctcagttgccaagaagcatcctaaaacttgggtacattacattgctgctgaagaggaggactgggactatgctcccttagtcctcgcccccgatgacagaagttataaaagtcaatatttgaacaatggccctcagcggattggtaggaagtacaaaaaagtccgatttatggcatacacagatgaaacctttaagactcgtgaagctattcagcatgaatcaggaatcttgggacctttactttatggggaagttggagacacactgttgattatatttaagaatcaagcaagcagaccatataacatctaccctcacggaatcactgatgtccgtcctttgtattcaaggagattaccaaaaggtgtaaaacatttgaaggattttccaattctgccaggagaaatattcaaatataaatggacagtgactgtagaagatgggccaactaaatcagatcctcggtgcctgacccgctattactctagtttcgttaatatggagagagatctagcttcaggactcattggccctctcctcatctgctacaaagaatctgtagatcaaagaggaaaccagataatgtcagacaagaggaatgtcatcctgttttctgtatttgatgagaaccgaagctggtacctcacagagaatatacaacgctttctccccaatccagctggagtgcagcttgaggatccagagttccaagcctccaacatcatgcacagcatcaatggctatgtttttgatagtttgcagttgtcagtttgtttgcatgaggtggcatactggtacattctaagcattggagcacagactgacttcctttctgtcttcttctctggatataccttcaaacacaaaatggtctatgaagacacactcaccctattcccattctcaggagaaactgtcttcatgtcgatggaaaacccaggtctatggattctggggtgccacaactcagactttcggaacagaggcatgaccgccttactgaaggtttctagttgtgacaagaacactggtgattattacgaggacagttatgaagatatttcagcatacttgctgagtaaaaacaatgccattgaaccaagaagcttctctcaaaacccaccagtcttgaaacgccatcaacgggaaataactcgtactactcttcagtcagatcaagaggaaattgactatgatgataccatatcagttgaaatgaagaaggaagattttgacatttatgatgaggatgaaaatcagagcccccgcagctttcaaaagaaaacacgacactattttattgctgcagtggagaggctctgggattatgggatgagtagctccccacatgttctaagaaacagggctcagagtggcagtgtccctcagttcaagaaagttgttttccaggaatttactgatggctcctttactcagcccttataccgtggagaactaaatgaacatttgggactcctggggccatatataagagcagaagttgaagataatatcatggtaactttcagaaatcaggcctctcgtccctattccttctattctagccttatttcttatgaggaagatcagaggcaaggagcagaacctagaaaaaactttgtcaagcctaatgaaaccaaaacttacttttggaaagtgcaacatcatatggcacccactaaagatgagtttgactgcaaagcctgggcttatttctctgatgttgacctggaaaaagatgtgcactcaggcctgattggaccccttctggtctgccacactaacacactgaaccctgctcatgggagacaagtgacagtacaggaatttgctctgtttttcaccatctttgatgagaccaaaagctggtacttcactgaaaatatggaaagaaactgcagggctccctgcaatatccagatggaagatcccacttttaaagagaattatcgcttccatgcaatcaatggctacataatggatacactacctggcttagtaatggctcaggatcaaaggattcgatggtatctgctcagcatgggcagcaatgaaaacatccattctattcatttcagtggacatgtgttcactgtacgaaaaaaagaggagtataaaatggcactgtacaatctctatccaggtgtttttgagacagtggaaatgttaccatccaaagctggaatttggcgggtggaatgccttattggcgagcatctacatgctgggatgagcacactttttctggtgtacagcaataagtgtcagactcccctgggaatggcttctggacacattagagattttcagattacagcttcaggacaatatggacagtgggccccaaagctggccagacttcattattccggatcaatcaatgcctggagcaccaaggagcccttttcttggatcaaggtggatctgttggcaccaatgattattcacggcatcaagacccagggtgcccgtcagaagttctccagcctctacatctctcagtttatcatcatgtatagtcttgatgggaagaagtggcagacttatcgaggaaattccactggaaccttaatggtcttctttggcaatgtggattcatctgggataaaacacaatatttttaaccctccaattattgctcgatacatccgtttgcacccaactcattatagcattcgcagcactcttcgcatggagttgatgggctgtgatttaaatagttgcagcatgccattgggaatggagagtaaagcaatatcagatgcacagattactgcttcatcctactttaccaatatgtttgccacctggtctccttcaaaagctcgacttcacctccaagggaggagtaatgcctggagacctcaggtgaataatccaaaagagtggctgcaagtggacttccagaagacaatgaaagtcacaggagtaactactcagggagtaaaatctctgcttaccagcatgtatgtgaaggagttcctcatctccagcagtcaagatggccatcagtggactctcttttttcagaatggcaaagtaaaggtttttcagggaaatcaagactccttcacacctgtggtgaactctctagacccaccgttactgactcgctaccttcgaattcacccccagagttgggtgcaccagattgccctgaggatggaggttctgggctgcgaggcacaggacctctacgacaaaactcacacatgcccaccgtgcccagctccagaactcctgggcggaccgtcagtcttcctcttccccccaaaacccaaggacaccctcatgatctcccggacccctgaggtcacatgcgtggtggtggacgtgagccacgaagaccctgaggtcaagttcaactggtacgtggacggcgtggaggtgcataatgccaagacaaagccgcgggaggagcagtacaacagcacgtaccgtgtggtcagcgtcctcaccgtcctgcaccaggactggctgaatggcaaggagtacaagtgcaaggtctccaacaaagccctcccagcccccatcgagaaaaccatctccaaagccaaagggcagccccgagaaccacaggtgtacaccctgcccccatcccgggatgagctgaccaagaaccaggtcagcctgacctgcctggtcaaaggcttctatcccagcgacatcgccgtggagtgggagagcaatgggcagccggagaacaactacaagaccacgcctcccgtgttggactccgacggctccttcttcctctacagcaagctcaccgtggacaagagcaggtggcagcaggggaacgtcttctcatgctccgtgatgcatgaggctctgcacaaccactacacgcagaagagcctctccctgtctccgggtaaa

SEQ ID NO: 2 - protein, 1684 aa, synthetic construct
  REGION 1..1684: note = B domain deleted FVIII-Fc chain
  REGION 1..19: note = MISC_FEATURE - Signal
  REGION 20..753: note = MISC_FEATURE - Heavy chain (HC)
  REGION 760..773: note = MISC_FEATURE - B domain
  REGION 1457..1684: note = MISC_FEATURE - Fc region
MQIELSTCFFLCLLRFCFSATRRYYLGAVELSWDYMQSDLGELPVDARFPPRVPKSFPFNTSVVYKKTLFVEFTDHLFNIAKPRPPWMGLLGPTIQAEVYDTVVITLKNMASHPVSLHAVGVSYWKASEGAEYDDQTSQREKEDDKVFPGGSHTYVWQVLKENGPMASDPLCLTYSYLSHVDLVKDLNSGLIGALLVCREGSLAKEKTQTLHKFILLFAVFDEGKSWHSETKNSLMQDRDAASARAWPKMHTVNGYVNRSLPGLIGCHRKSVYWHVIGMGTTPEVHSIFLEGHTFLVRNHRQASLEISPITFLTAQTLLMDLGQFLLFCHISSHQHDGMEAYVKVDSCPEEPQLRMKNNEEAEDYDDDLTDSEMDVVRFDDDNSPSFIQIRSVAKKHPKTWVHYIAAEEEDWDYAPLVLAPDDRSYKSQYLNNGPQRIGRKYKKVRFMAYTDETFKTREAIQHESGILGPLLYGEVGDTLLIIFKNQASRPYNIYPHGITDVRPLYSRRLPKGVKHLKDFPILPGEIFKYKWTVTVEDGPTKSDPRCLTRYYSSFVNMERDLASGLIGPLLICYKESVDQRGNQIMSDKRNVILFSVFDENRSWYLTENIQRFLPNPAGVQLEDPEFQASNIMHSINGYVFDSLQLSVCLHEVAYWYILSIGAQTDFLSVFFSGYTFKHKMVYEDTLTLFPFSGETVFMSMENPGLWILGCHNSDFRNRGMTALLKVSSCDKNTGDYYEDSYEDISAYLLSKNNAIEPRSFSQNPPVLKRHQREITRTTLQSDQEEIDYDDTISVEMKKEDFDIYDEDENQSPRSFQKKTRHYFIAAVERLWDYGMSSSPHVLRNRAQSGSVPQFKKVVFQEFTDGSFTQPLYRGELNEHLGLLGPYIRAEVEDNIMVTFRNQASRPYSFYSSLISYEEDQRQGAEPRKNFVKPNETKTYFWKVQHHMAPTKDEFDCKAWAYFSDVDLEKDVHSGLIGPLLVCHTNTLNPAHGRQVTVQEFALFFTIFDETKSWYFTENMERNCRAPCNIQMEDPTFKENYRFHAINGYIMDTLPGLVMAQDQRIRWYLLSMGSNENIHSIHFSGHVFTVRKKEEYKMALYNLYPGVFETVEMLPSKAGIWRVECLIGEHLHAGMSTLFLVYSNKCQTPLGMASGHIRDFQITASGQYGQWAPKLARLHYSGSINAWSTKEPFSWIKVDLLAPMIIHGIKTQGARQKFSSLYISQFIIMYSLDGKKWQTYRGNSTGTLMVFFGNVDSSGIKHNIFNPPIIARYIRLHPTHYSIRSTLRMELMGCDLNSCSMPLGMESKAISDAQITASSYFTNMFATWSPSKARLHLQGRSNAWRPQVNNPKEWLQVDFQKTMKVTGVTTQGVKSLLTSMYVKEFLISSSQDGHQWTLFFQNGKVKVFQGNQDSFTPVVNSLDPPLLTRYLRIHPQSWVHQIALRMEVLGCEAQDLYDKTHTCPPCPAPELLGGPSVFLFPPKPKDTLMISRTPEVTCVVVDVSHEDPEVKFNWYVDGVEVHNAKTKPREEQYNSTYRVVSVLTVLHQDWLNGKEYKCKVSNKALPAPIEKTISKAKGQPREPQVYTLPPSRDELTKNQVSLTCLVKGFYPSDIAVEWESNGQPENNYKTTPPVLDSDGSFFLYSKLTVDKSRWQQGNVFSCSVMHEALHNHYTQKSLSLSPGK

SEQ ID NO: 3 - DNA, 741 bp, synthetic construct
  misc_feature 1..741: note = Fc region
  regulatory 1..60: note = Mouse Ig kappa signal; regulatory_class = other
  source 1..741: mol_type = other DNA
atggagacagacacactcctgctatgggtactgctgctctgggttccaggttccactggtgacaaaactcacacatgcccaccgtgcccagcacctgaactcctgggaggaccgtcagtcttcctcttccccccaaaacccaaggacaccctcatgatctcccggacccctgaggtcacatgcgtggtggtggacgtgagccacgaagaccctgaggtcaagttcaactggtacgtggacggcgtggaggtgcataatgccaagacaaagccgcgggaggagcagtacaacagcacgtaccgtgtggtcagcgtcctcaccgtcctgcaccaggactggctgaatggcaaggagtacaagtgcaaggtctccaacaaagccctcccagcccccatcgagaaaaccatctccaaagccaaagggcagccccgagaaccacaggtgtacaccctgcccccatcccgcgatgagctgaccaagaaccaggtcagcctgacctgcctggtcaaaggcttctatcccagcgacatcgccgtggagtgggagagcaatgggcagccggagaacaactacaagaccacgcctcccgtgttggactccgacggctccttcttcctctacagcaagctcaccgtggacaagagcaggtggcagcaggggaacgtcttctcatgctccgtgatgcatgaggctctgcacaaccactacacgcagaagagcctctccctgtctccgggtaaa

SEQ ID NO: 4 - protein, 247 aa, synthetic construct
  REGION 1..247: note = Fc chain
  REGION 1..20: note = MISC_FEATURE - heterologous signal from Mouse Ig kappa chain
METDTLLLWVLLLWVPGSTGDKTHTCPPCPAPELLGGPSVFLFPPKPKDTLMISRTPEVTCVVVDVSHEDPEVKFNWYVDGVEVHNAKTKPREEQYNSTYRVVSVLTVLHQDWLNGKEYKCKVSNKALPAPIEKTISKAKGQPREPQVYTLPPSRDELTKNQVSLTCLVKGFYPSDIAVEWESNGQPENNYKTTPPVLDSDGSFFLYSKLTVDKSRWQQGNVFSCSVMHEALHNHYTQKSLSLSPGK

SEQ ID NO: 5 - DNA, 7734 bp, synthetic construct
  misc_feature 1..7734: note = Full length FVIIIFc
  regulatory 1..57: note = FVIII signal; regulatory_class = other
  misc_feature 7054..7734: note = Fc region
  source 1..7734: mol_type = other DNA
atgcaaatagagctctccacctgcttctttctgtgccttttgcgattctgctttagtgccaccagaagatactacctgggtgcagtggaactgtcatgggactatatgcaaagtgatctcggtgagctgcctgtggacgcaagatttcctcctagagtgccaaaatcttttccattcaacacctcagtcgtgtacaaaaagactctgtttgtagaattcacggatcaccttttcaacatcgctaagccaaggccaccctggatgggtctgctaggtcctaccatccaggctgaggtttatgatacagtggtcattacacttaagaacatggcttcccatcctgtcagtcttcatgctgttggtgtatcctactggaaagcttctgagggagctgaatatgatgatcagaccagtcaaagggagaaagaagatgataaagtcttccctggtggaagccatacatatgtctggcaggtcctgaaagagaatggtccaatggcctctgacccactgtgccttacctactcatatctttctcatgtggacctggtaaaagacttgaattcaggcctcattggagccctactagtatgtagagaagggagtctggccaaggaaaagacacagaccttgcacaaatttatactactttttgctgtatttgatgaagggaaaagttggcactcagaaacaaagaactccttgatgcaggatagggatgctgcatctgctcgggcctggcctaaaatgcacacagtcaatggttatgtaaacaggtctctgccaggtctgattggatgccacaggaaatcagtctattggcatgtgattggaatgggcaccactcctgaagtgcactcaatattcctcgaaggtcacacatttcttgtgaggaaccatcgccaggcgtccttggaaatctcgccaataactttccttactgctcaaacactcttgatggaccttggacagtttctactgttttgtcatatctcttcccaccaacatgatggcatggaagcttatgtcaaagtagacagctgtccagaggaaccccaactacgaatgaaaaataatgaagaagcggaagactatgatgatgatcttactgattctgaaatggatgtggtcaggtttgatgatgacaactctccttcctttatccaaattcgctcagttgccaagaagcatcctaaaacttgggtacattacattgctgctgaagaggaggactgggactatgctcccttagtcctcgcccccgatgacagaagttataaaagtcaatatttgaacaatggccctcagcggattggtaggaagtacaaaaaagtccgatttatggcatacacagatgaaacctttaagactcgtgaagctattcagcatgaatcaggaatcttgggacctttactttatggggaagttggagacacactgttgattatatttaagaatcaagcaagcagaccatataacatctaccctcacggaatcactgatgtccgtcctttgtattcaaggagattaccaaaaggtgtaaaacatttgaaggattttccaattctgccaggagaaatattcaaatataaatggacagtgactgtagaagatgggccaactaaatcagatcctcggtgcctgacccgctattactctagtttcgttaatatggagagagatctagcttcaggactcattggccctctcctcatctgctacaaagaatctgtagatcaaagaggaaaccagataatgtcagacaagaggaatgtcatcctgttttctgtatttgatgagaaccgaagctggtacctcacagagaatatacaacgctttctccccaatccagctggagtgcagcttgaggatccagagttccaagcctccaacatcatgcacagcatcaatggctatgtttttgatagtttgcagttgtcagtttgtttgcatgaggtggcatactggtacattctaagcattggagcacagactgacttcctttctgtcttcttctctggatataccttcaaacacaaaatggtctatgaagacacactcaccctattcccattctcaggagaaactgtcttcatgtcgatggaaaacccaggtctatggattctggggtgccacaactcagactttcggaacagaggcatgaccgccttactgaaggtttctagttgtgacaagaacactggtgattattacgaggacagttatgaagatatttcagcatacttgctgagtaaaaacaatgccattgaaccaagaagcttctcccagaattcaagacaccctagcactaggcaaaagcaatttaatgccaccacaattccagaaaatgacatagagaagactgacccttggtttgcacacagaacacctatgcctaaaatacaaaatgtctcctctagtgatttgttgatgctcttgcgacagagtcctactccacatgggctatccttatctgatctccaagaagccaaatatgagactttttctgatgatccatcacctggagcaatagacagtaataacagcctgtctgaaatgacacacttcaggccacagctccatcacagtggggacatggtatttacccctgagtcaggcctccaattaagattaaatgagaaactggggacaactgcagcaacagagttgaagaaacttgatttcaaagtttctagtacatcaaataatctgatttcaacaattccatcagacaatttggcagcaggtactgataatacaagttccttaggacccccaagtatgccagttcattatgatagtcaattagataccactctatttggcaaaaagtcatctccccttactgagtctggtggacctctgagcttgagtgaagaaaataatgattcaaagttgttagaatcaggtttaatgaatagccaagaaagttcatggggaaaaaatgtatcgtcaacagagagtggtaggttatttaaagggaaaagagctcatggacctgctttgttgactaaagataatgccttattcaaagttagcatctctttgttaaagacaaacaaaacttccaataattcagcaactaatagaaagactcacattgatggcccatcattattaattgagaatagtccatcagtctggcaaaatatattagaaagtgacactgagtttaaaaaagtgacacctttgattcatgacagaatgcttatggacaaaaatgctacagctttgaggctaaatcatatgtcaaataaaactacttcatcaaaaaacatggaaatggtccaacagaaaaaagagggccccattccaccagatgcacaaaatccagatatgtcgttctttaagatgctattcttgccagaatcagcaaggtggatacaaaggactcatggaaagaactctctgaactctgggcaaggccccagtccaaagcaattagtatccttaggaccagaaaaatctgtggaaggtcagaatttcttgtctgagaaaaacaaagtggtagtaggaaagggtgaatttacaaaggacgtaggactcaaagagatggtttttccaagcagcagaaacctatttcttactaacttggataatttacatgaaaataatacacacaatcaagaaaaaaaaattcaggaagaaatagaaaagaaggaaacattaatccaagagaatgtagttttgcctcagatacatacagtgactggcactaagaatttcatgaagaaccttttcttactgagcactaggcaaaatgtagaaggttcatatgacggggcatatgctccagtacttcaagattttaggtcattaaatgattcaacaaatagaacaaagaaacacacagctcatttctcaaaaaaaggggaggaagaaaacttggaaggcttgggaaatcaaaccaagcaaattgtagagaaatatgcatgcaccacaaggatatctcctaatacaagccagcagaattttgtcacgcaacgtagtaagagagctttgaaacaattcagactcccactagaagaaacagaacttgaaaaaaggataattgtggatgacacctcaacccagtggtccaaaaacatgaaacatttgaccccgagcaccctcacacagatagactacaatgagaaggagaaaggggccattactcagtctcccttatcagattgccttacgaggagtcatagcatccctcaagcaaatagatctccattacccattgcaaaggtatcatcatttccatctattagacctatatatctgaccagggtcctattccaagacaactcttctcatcttccagcagcatcttatagaaagaaagattctggggtccaagaaagcagtcatttcttacaaggagccaaaaaaaataacctttctttagccattctaaccttggagatgactggtgatcaaagagaggttggctccctggggacaagtgccacaaattcagtcacatacaagaaagttgagaacactgttctcccgaaaccagacttgcccaaaacatctggcaaagttgaattgcttccaaaagttcacatttatcagaaggacctattccctacggaaactagcaatgggtctcctggccatctggatctcgtggaagggagccttcttcagggaacagagggagcgattaagtggaatgaagcaaacagacctggaaaagttccctttctgagagtagcaacagaaagctctgcaaagactccctccaagctattggatcctcttgcttgggataaccactatggtactcagataccaaaagaagagtggaaatcccaagagaagtcaccagaaaaaacagcttttaagaaaaaggataccattttgtccctgaacgcttgtgaaagcaatcatgcaatagcagcaataaatgagggacaaaataagcccgaaatagaagtcacctgggcaaagcaaggtaggactgaaaggctgtgctctcaaaacccaccagtcttgaaacgccatcaacgggaaataactcgtactactcttcagtcagatcaagaggaaattgactatgatgataccatatcagttgaaatgaagaaggaagattttgacatttatgatgaggatgaaaatcagagcccccgcagctttcaaaagaaaacacgacactattttattgctgcagtggagaggctctgggattatgggatgagtagctccccacatgttctaagaaacagggctcagagtggcagtgtccctcagttcaagaaagttgttttccaggaatttactgatggctcctttactcagcccttataccgtggagaactaaatgaacatttgggactcctggggccatatataagagcagaagttgaagataatatcatggtaactttcagaaatcaggcctctcgtccctattccttctattctagccttatttcttatgaggaagatcagaggcaaggagcagaacctagaaaaaactttgtcaagcctaatgaaaccaaaacttacttttggaaagtgcaacatcatatggcacccactaaagatgagtttgactgcaaagcctgggcttatttctctgatgttgacctggaaaaagatgtgcactcaggcctgattggaccccttctggtctgccacactaacacactgaaccctgctcatgggagacaagtgacagtacaggaatttgctctgtttttcaccatctttgatgagaccaaaagctggtacttcactgaaaatatggaaagaaactgcagggctccctgcaatatccagatggaagatcccacttttaaagagaattatcgcttccatgcaatcaatggctacataatggatacactacctggcttagtaatggctcaggatcaaaggattcgatggtatctgctcagcatgggcagcaatgaaaacatccattctattcatttcagtggacatgtgttcactgtacgaaaaaaagaggagtataaaatggcactgtacaatctctatccaggtgtttttgagacagtggaaatgttaccatccaaagctggaatttggcgggtggaatgccttattggcgagcatctacatgctgggatgagcacactttttctggtgtacagcaataagtgtcagactcccctgggaatggcttctggacacattagagattttcagattacagcttcaggacaatatggacagtgggccccaaagctggccagacttcattattccggatcaatcaatgcctggagcaccaaggagcccttttcttggatcaaggtggatctgttggcaccaatgattattcacggcatcaagacccagggtgcccgtcagaagttctccagcctctacatctctcagtttatcatcatgtatagtcttgatgggaagaagtggcagacttatcgaggaaattccactggaaccttaatggtcttctttggcaatgtggattcatctgggataaaacacaatatttttaaccctccaattattgctcgatacatccgtttgcacccaactcattatagcattcgcagcactcttcgcatggagttgatgggctgtgatttaaatagttgcagcatgccattgggaatggagagtaaagcaatatcagatgcacagattactgcttcatcctactttaccaatatgtttgccacctggtctccttcaaaagctcgacttcacctccaagggaggagtaatgcctggagacctcaggtgaataatccaaaagagtggctgcaagtggacttccagaagacaatgaaagtcacaggagtaactactcagggagtaaaatctctgcttaccagcatgtatgtgaaggagttcctcatctccagcagtcaagatggccatcagtggactctcttttttcagaatggcaaagtaaaggtttttcagggaaatcaagactccttcacacctgtggtgaactctctagacccaccgttactgactcgctaccttcgaattcacccccagagttgggtgcaccagattgccctgaggatggaggttctgggctgcgaggcacaggacctctacgacaaaactcacacatgcccaccgtgcccagctccagaactcctgggcggaccgtcagtcttcctcttccccccaaaacccaaggacaccctcatgatctcccggacccctgaggtcacatgcgtggtggtggacgtgagccacgaagaccctgaggtcaagttcaactggtacgtggacggcgtggaggtgcataatgccaagacaaagccgcgggaggagcagtacaacagcacgtaccgtgtggtcagcgtcctcaccgtcctgcaccaggactggctgaatggcaaggagtacaagtgcaaggtctccaacaaagccctcccagcccccatcgagaaaaccatctccaaagccaaagggcagccccgagaaccacaggtgtacaccctgcccccatcccgggatgagctgaccaagaaccaggtcagcctgacctgcctggtcaaaggcttctatcccagcgacatcgccgtggagtgggagagcaatgggcagccggagaacaactacaagaccacgcctcccgtgttggactccgacggctccttcttcctctacagcaagctcaccgtggacaagagcaggtggcagcaggggaacgtcttctcatgctccgtgatgcatgaggctctgcacaaccactacacgcagaagagcctctccctgtctccgggtaaa

SEQ ID NO: 6 - protein, 2578 aa, synthetic construct
  REGION 1..2578: note = Full length FVIIIFc chain
  REGION 1..19: note = MISC_FEATURE - FVIII signal
  REGION 20..759: note = MISC_FEATURE - HC
  REGION 760..1667: note = MISC_FEATURE - B domain
  REGION 2352..2578: note = MISC_FEATURE - Fc region
MQIELSTCFFLCLLRFCFSATRRYYLGAVELSWDYMQSDLGELPVDARFPPRVPKSFPFNTSVVYKKTLFVEFTDHLFNIAKPRPPWMGLLGPTIQAEVYDTVVITLKNMASHPVSLHAVGVSYWKASEGAEYDDQTSQREKEDDKVFPGGSHTYVWQVLKENGPMASDPLCLTYSYLSHVDLVKDLNSGLIGALLVCREGSLAKEKTQTLHKFILLFAVFDEGKSWHSETKNSLMQDRDAASARAWPKMHTVNGYVNRSLPGLIGCHRKSVYWHVIGMGTTPEVHSIFLEGHTFLVRNHRQASLEISPITFLTAQTLLMDLGQFLLFCHISSHQHDGMEAYVKVDSCPEEPQLRMKNNEEAEDYDDDLTDSEMDVVRFDDDNSPSFIQIRSVAKKHPKTWVHYIAAEEEDWDYAPLVLAPDDRSYKSQYLNNGPQRIGRKYKKVRFMAYTDETFKTREAIQHESGILGPLLYGEVGDTLLIIFKNQASRPYNIYPHGITDVRPLYSRRLPKGVKHLKDFPILPGEIFKYKWTVTVEDGPTKSDPRCLTRYYSSFVNMERDLASGLIGPLLICYKESVDQRGNQIMSDKRNVILFSVFDENRSWYLTENIQRFLPNPAGVQLEDPEFQASNIMHSINGYVFDSLQLSVCLHEVAYWYILSIGAQTDFLSVFFSGYTFKHKMVYEDTLTLFPFSGETVFMSMENPGLWILGCHNSDFRNRGMTALLKVSSCDKNTGDYYEDSYEDISAYLLSKNNAIEPRSFSQNSRHPSTRQKQFNATTIPENDIEKTDPWFAHRTPMPKIQNVSSSDLLMLLRQSPTPHGLSLSDLQEAKYETFSDDPSPGAIDSNNSLSEMTHFRPQLHHSGDMVFTPESGLQLRLNEKLGTTAATELKKLDFKVSSTSNNLISTIPSDNLAAGTDNTSSLGPPSMPVHYDSQLDTTLFGKKSSPLTESGGPLSLSEENNDSKLLESGLMNSQESSWGKNVSSTESGRLFKGKRAHGPALLTKDNALFKVSISLLKTNKTSNNSATNRKTHIDGPSLLIENSPSVWQNILESDTEFKKVTPLIHDRMLMDKNATALRLNHMSNKTTSSKNMEMVQQKKEGPIPPDAQNPDMSFFKMLFLPESARWIQRTHGKNSLNSGQGPSPKQLVSLGPEKSVEGQNFLSEKNKVVVGKGEFTKDVGLKEMVFPSSRNLFLTNLDNLHENNTHNQEKKIQEEIEKKETLIQENVVLPQIHTVTGTKNFMKNLFLLSTRQNVEGSYDGAYAPVLQDFRSLNDSTNRTKKHTAHFSKKGEEENLEGLGNQTKQIVEKYACTTRISPNTSQQNFVTQRSKRALKQFRLPLEETELEKRIIVDDTSTQWSKNMKHLTPSTLTQIDYNEKEKGAITQSPLSDCLTRSHSIPQANRSPLPIAKVSSFPSIRPIYLTRVLFQDNSSHLPAASYRKKDSGVQESSHFLQGAKKNNLSLAILTLEMTGDQREVGSLGTSATNSVTYKKVENTVLPKPDLPKTSGKVELLPKVHIYQKDLFPTETSNGSPGHLDLVEGSLLQGTEGAIKWNEANRPGKVPFLRVATESSAKTPSKLLDPLAWDNHYGTQIPKEEWKSQEKSPEKTAFKKKDTILSLNACESNHAIAAINEGQNKPEIEVTWAKQGRTERLCSQNPPVLKRHQREITRTTLQSDQEEIDYDDTISVEMKKEDFDIYDEDENQSPRSFQKKTRHYFIAAVERLWDYGMSSSPHVLRNRAQSGSVPQFKKVVFQEFTDGSFTQPLYRGELNEHLGLLGPYIRAEVEDNIMVTFRNQASRPYSFYSSLISYEEDQRQGAEPRKNFVKPNETKTYFWKVQHHMAPTKDEFDCKAWAYFSDVDLEKDVHSGLIGPLLVCHTNTLNPAHGRQVTVQEFALFFTIFDETKSWYFTENMERNCRAPCNIQMEDPTFKENYRFHAINGYIMDTLPGLVMAQDQRIRWYLLSMGSNENIHSIHFSGHVFTVRKKEEYKMALYNLYPGVFETVEMLPSKAGIWRVECLIGEHLHAGMSTLFLVYSNKCQTPLGMASGHIRDFQITASGQYGQWAPKLARLHYSGSINAWSTKEPFSWIKVDLLAPMIIHGIKTQGARQKFSSLYISQFIIMYSLDGKKWQTYRGNSTGTLMVFFGNVDSSGIKHNIFNPPIIARYIRLHPTHYSIRSTLRMELMGCDLNSCSMPLGMESKAISDAQITASSYFTNMFATWSPSKARLHLQGRSNAWRPQVNNPKEWLQVDFQKTMKVTGVTTQGVKSLLTSMYVKEFLISSSQDGHQWTLFFQNGKVKVFQGNQDSFTPVVNSLDPPLLTRYLRIHPQSWVHQIALRMEVLGCEAQDLYDKTHTCPPCPAPELLGGPSVFLFPPKPKDTLMISRTPEVTCVVVDVSHEDPEVKFNWYVDGVEVHNAKTKPREEQYNSTYRVVSVLTVLHQDWLNGKEYKCKVSNKALPAPIEKTISKAKGQPREPQVYTLPPSRDELTKNQVSLTCLVKGFYPSDIAVEWESNGQPENNYKTTPPVLDSDGSFFLYSKLTVDKSRWQQGNVFSCSVMHEALHNHYTQKSLSLSPGK

SEQ ID NO: 7 - DNA, 2958 bp, synthetic construct
  misc_feature 1..2958: note = Heavy Chain (HC)-Fc
  misc_feature 1..57: note = Signal
  misc_feature 2278..2958: note = Fc region
  source 1..2958: mol_type = other DNA
atgcaaatagagctctccacctgcttctttctgtgccttttgcgattctgctttagtgccaccagaagatactacctgggtgcagtggaactgtcatgggactatatgcaaagtgatctcggtgagctgcctgtggacgcaagatttcctcctagagtgccaaaatcttttccattcaacacctcagtcgtgtacaaaaagactctgtttgtagaattcacggatcaccttttcaacatcgctaagccaaggccaccctggatgggtctgctaggtcctaccatccaggctgaggtttatgatacagtggtcattacacttaagaacatggcttcccatcctgtcagtcttcatgctgttggtgtatcctactggaaagcttctgagggagctgaatatgatgatcagaccagtcaaagggagaaagaagatgataaagtcttccctggtggaagccatacatatgtctggcaggtcctgaaagagaatggtccaatggcctctgacccactgtgccttacctactcatatctttctcatgtggacctggtaaaagacttgaattcaggcctcattggagccctactagtatgtagagaagggagtctggccaaggaaaagacacagaccttgcacaaatttatactactttttgctgtatttgatgaagggaaaagttggcactcagaaacaaagaactccttgatgcaggatagggatgctgcatctgctcgggcctggcctaaaatgcacacagtcaatggttatgtaaacaggtctctgccaggtctgattggatgccacaggaaatcagtctattggcatgtgattggaatgggcaccactcctgaagtgcactcaatattcctcgaaggtcacacatttcttgtgaggaaccatcgccaggcgtccttggaaatctcgccaataactttccttactgctcaaacactcttgatggaccttggacagtttctactgttttgtcatatctcttcccaccaacatgatggcatggaagcttatgtcaaagtagacagctgtccagaggaaccccaactacgaatgaaaaataatgaagaagcggaagactatgatgatgatcttactgattctgaaatggatgtggtcaggtttgatgatgacaactctccttcctttatccaaattcgctcagttgccaagaagcatcctaaaacttgggtacattacattgctgctgaagaggaggactgggactatgctcccttagtcctcgcccccgatgacagaagttataaaagtcaatatttgaacaatggccctcagcggattggtaggaagtacaaaaaagtccgatttatggcatacacagatgaaacctttaagactcgtgaagctattcagcatgaatcaggaatcttgggacctttactttatggggaagttggagacacactgttgattatatttaagaatcaagcaagcagaccatataacatctaccctcacggaatcactgatgtccgtcctttgtattcaaggagattaccaaaaggtgtaaaacatttgaaggattttccaattctgccaggagaaatattcaaatataaatggacagtgactgtagaagatgggccaactaaatcagatcctcggtgcctgacccgctattactctagtttcgttaatatggagagagatctagcttcaggactcattggccctctcctcatctgctacaaagaatctgtagatcaaagaggaaaccagataatgtcagacaagaggaatgtcatcctgttttctgtatttgatgagaaccgaagctggtacctcacagagaatatacaacgctttctccccaatccagctggagtgcagcttgaggatccagagttccaagcctccaacatcatgcacagcatcaatggctatgtttttgatagtttgcagttgtcagtttgtttgcatgaggtggcatactggtacattctaagcattggagcacagactgacttcctttctgtcttcttctctggatataccttcaaacacaaaatggtctatgaagacacactcaccctattcccattctcaggagaaactgtcttcatgtcgatggaaaacccaggtctatggattctggggtgccacaactcagactttcggaacagaggcatgaccgccttactgaaggtttctagttgtgacaagaacactggtgattattacgaggacagttatgaagatatttcagcatacttgctgagtaaaaacaatgccattgaaccaagagacaaaactcacacatgcccaccgtgcccagctccagaactcctgggcggaccgtcagtcttcctcttccccccaaaacccaaggacaccctcatgatctcccggacccctgaggtcacatgcgtggtggtggacgtgagccacgaagaccctgaggtcaagttcaactggtacgtggacggcgtggaggtgcataatgccaagacaaagccgcgggaggagcagtacaacagcacgtaccgtgtggtcagcgtcctcaccgtcctgcaccaggactggctgaatggcaaggagtacaagtgcaaggtctccaacaaagccctcccagcccccatcgagaaaaccatctccaaagccaaagggcagccccgagaaccacaggtgtacaccctgcccccatcccgggatgagctgaccaagaaccaggtcagcctgacctgcctggtcaaaggcttctatcccagcgacatcgccgtggagtgggagagcaatgggcagccggagaacaactacaagaccacgcctcccgtgttggactccgacggctccttcttcctctacagcaagctcaccgtggacaagagcaggtggcagcaggggaacgtcttctcatgctccgtgatgcatgaggctctgcacaaccactacacgcagaagagcctctccctgtctccgggtaaa

SEQ ID NO: 8 - protein, 986 aa, synthetic construct
  REGION 1..986: note = HC-Fc
  REGION 1..19: note = MISC_FEATURE - Signal
  REGION 760..986: note = MISC_FEATURE - Fc region
MQIELSTCFFLCLLRFCFSATRRYYLGAVELSWDYMQSDLGELPVDARFPPRVPKSFPFNTSVVYKKTLFVEFTDHLFNIAKPRPPWMGLLGPTIQAEVYDTVVITLKNMASHPVSLHAVGVSYWKASEGAEYDDQTSQREKEDDKVFPGGSHTYVWQVLKENGPMASDPLCLTYSYLSHVDLVKDLNSGLIGALLVCREGSLAKEKTQTLHKFILLFAVFDEGKSWHSETKNSLMQDRDAASARAWPKMHTVNGYVNRSLPGLIGCHRKSVYWHVIGMGTTPEVHSIFLEGHTFLVRNHRQASLEISPITFLTAQTLLMDLGQFLLFCHISSHQHDGMEAYVKVDSCPEEPQLRMKNNEEAEDYDDDLTDSEMDVVRFDDDNSPSFIQIRSVAKKHPKTWVHYIAAEEEDWDYAPLVLAPDDRSYKSQYLNNGPQRIGRKYKKVRFMAYTDETFKTREAIQHESGILGPLLYGEVGDTLLIIFKNQASRPYNIYPHGITDVRPLYSRRLPKGVKHLKDFPILPGEIFKYKWTVTVEDGPTKSDPRCLTRYYSSFVNMERDLASGLIGPLLICYKESVDQRGNQIMSDKRNVILFSVFDENRSWYLTENIQRFLPNPAGVQLEDPEFQASNIMHSINGYVFDSLQLSVCLHEVAYWYILSIGAQTDFLSVFFSGYTFKHKMVYEDTLTLFPFSGETVFMSMENPGLWILGCHNSDFRNRGMTALLKVSSCDKNTGDYYEDSYEDISAYLLSKNNAIEPRDKTHTCPPCPAPELLGGPSVFLFPPKPKDTLMISRTPEVTCVVVDVSHEDPEVKFNWYVDGVEVHNAKTKPREEQYNSTYRVVSVLTVLHQDWLNGKEYKCKVSNKALPAPIEKTISKAKGQPREPQVYTLPPSRDELTKNQVSLTCLVKGFYPSDIAVEWESNGQPENNYKTTPPVLDSDGSFFLYSKLTVDKSRWQQGNVFSCSVMHEALHNHYTQKSLSLSPGK

SEQ ID NO: 9 - DNA, 2973 bp, synthetic construct
  misc_feature 1..2973: note = Heavy Chain (HC)-Fc (5 amino acid linker between HC and Fc)
  regulatory 1..57: note = Signal; regulatory_class = other
  misc_feature 2278..2292: note = 5 amino acid linker
  misc_feature 2293..2973: note = Fc region
  source 1..2973: mol_type = other DNA
atgcaaatagagctctccacctgcttctttctgtgccttttgcgattctgctttagtgccaccagaagatactacctgggtgcagtggaactgtcatgggactatatgcaaagtgatctcggtgagctgcctgtggacgcaagatttcctcctagagtgccaaaatcttttccattcaacacctcagtcgtgtacaaaaagactctgtttgtagaattcacggatcaccttttcaacatcgctaagccaaggccaccctggatgggtctgctaggtcctaccatccaggctgaggtttatgatacagtggtcattacacttaagaacatggcttcccatcctgtcagtcttcatgctgttggtgtatcctactggaaagcttctgagggagctgaatatgatgatcagaccagtcaaagggagaaagaagatgataaagtcttccctggtggaagccatacatatgtctggcaggtcctgaaagagaatggtccaatggcctctgacccactgtgccttacctactcatatctttctcatgtggacctggtaaaagacttgaattcaggcctcattggagccctactagtatgtagagaagggagtctggccaaggaaaagacacagaccttgcacaaatttatactactttttgctgtatttgatgaagggaaaagttggcactcagaaacaaagaactccttgatgcaggatagggatgctgcatctgctcgggcctggcctaaaatgcacacagtcaatggttatgtaaacaggtctctgccaggtctgattggatgccacaggaaatcagtctattggcatgtgattggaatgggcaccactcctgaagtgcactcaatattcctcgaaggtcacacatttcttgtgaggaaccatcgccaggcgtccttggaaatctcgccaataactttccttactgctcaaacactcttgatggaccttggacagtttctactgttttgtcatatctcttcccaccaacatgatggcatggaagcttatgtcaaagtagacagctgtccagaggaaccccaactacgaatgaaaaataatgaagaagcggaagactatgatgatgatcttactgattctgaaatggatgtggtcaggtttgatgatgacaactctccttcctttatccaaattcgctcagttgccaagaagcatcctaaaacttgggtacattacattgctgctgaagaggaggactgggactatgctcccttagtcctcgcccccgatgacagaagttataaaagtcaatatttgaacaatggccctcagcggattggtaggaagtacaaaaaagtccgatttatggcatacacagatgaaacctttaagactcgtgaagctattcagcatgaatcaggaatcttgggacctttactttatggggaagttggagacacactgttgattatatttaagaatcaagcaagcagaccatataacatctaccctcacggaatcactgatgtccgtcctttgtattcaaggagattaccaaaaggtgtaaaacatttgaaggattttccaattctgccaggagaaatattcaaatataaatggacagtgactgtagaagatgggccaactaaatcagatcctcggtgcctgacccgctattactctagtttcgttaatatggagagagatctagcttcaggactcattggccctctcctcatctgctacaaagaatctgtagatcaaagaggaaaccagataatgtcagacaagaggaatgtcatcctgttttctgtatttgatgagaaccgaagctggtacctcacagagaatatacaacgctttctccccaatccagctggagtgcagcttgaggatccagagttccaagcctccaacatcatgcacagcatcaatggctatgtttttgatagtttgcagttgtcagtttgtttgcatgaggtggcatactggtacattctaagcattggagcacagactgacttcctttctgtcttcttctctggatataccttcaaacacaaaatggtctatgaagacacactcaccctattcccattctcaggagaaactgtcttcatgtcgatggaaaacccaggtctatggattctggggtgccacaactcagactttcggaacagaggcatgaccgccttactgaaggtttctagttgtgacaagaacactggtgattattacgaggacagttatgaagatatttcagcatacttgctgagtaaaaacaatgccattgaaccaagaagcttctcccagaatgacaaaactcacacatgcccaccgtgcccagctccagaactcctgggcggaccgtcagtcttcctcttccccccaaaacccaaggacaccctcatgatctcccggacccctgaggtcacatgcgtggtggtggacgtgagccacgaagaccctgaggtcaagttcaactggtacgtggacggcgtggaggtgcataatgccaagacaaagccgcgggaggagcagtacaacagcacgtaccgtgtggtcagcgtcctcaccgtcctgcaccaggactggctgaatggcaaggagtacaagtgcaaggtctccaacaaagccctcccagcccccatcgagaaaaccatctccaaagccaaagggcagccccgagaaccacaggtgtacaccctgcccccatcccgggatgagctgaccaagaaccaggtcagcctgacctgcctggtcaaaggcttctatcccagcgacatcgccgtggagtgggagagcaatgggcagccggagaacaactacaagaccacgcctcccgtgttggactccgacggctccttcttcctctacagcaagctcaccgtggacaagagcaggtggcagcaggggaacgtcttctcatgctccgtgatgcatgaggctctgcacaaccactacacgcagaagagcctctccctgtctccgggtaaa

SEQ ID NO: 10 - protein, 991 aa, synthetic construct
  REGION 1..991: note = HC+5-Fc
  REGION 1..19: note = MISC_FEATURE - Signal
  REGION 760..764: note = MISC_FEATURE - B domain
  REGION 765..991: note = MISC_FEATURE - Fc region
MQIELSTCFFLCLLRFCFSATRRYYLGAVELSWDYMQSDLGELPVDARFPPRVPKSFPFNTSVVYKKTLFVEFTDHLFNIAKPRPPWMGLLGPTIQAEVYDTVVITLKNMASHPVSLHAVGVSYWKASEGAEYDDQTSQREKEDDKVFPGGSHTYVWQVLKENGPMASDPLCLTYSYLSHVDLVKDLNSGLIGALLVCREGSLAKEKTQTLHKFILLFAVFDEGKSWHSETKNSLMQDRDAASARAWPKMHTVNGYVNRSLPGLIGCHRKSVYWHVIGMGTTPEVHSIFLEGHTFLVRNHRQASLEISPITFLTAQTLLMDLGQFLLFCHISSHQHDGMEAYVKVDSCPEEPQLRMKNNEEAEDYDDDLTDSEMDVVRFDDDNSPSFIQIRSVAKKHPKTWVHYIAAEEEDWDYAPLVLAPDDRSYKSQYLNNGPQRIGRKYKKVRFMAYTDETFKTREAIQHESGILGPLLYGEVGDTLLIIFKNQASRPYNIYPHGITDVRPLYSRRLPKGVKHLKDFPILPGEIFKYKWTVTVEDGPTKSDPRCLTRYYSSFVNMERDLASGLIGPLLICYKESVDQRGNQIMSDKRNVILFSVFDENRSWYLTENIQRFLPNPAGVQLEDPEFQASNIMHSINGYVFDSLQLSVCLHEVAYWYILSIGAQTDFLSVFFSGYTFKHKMVYEDTLTLFPFSGETVFMSMENPGLWILGCHNSDFRNRGMTALLKVSSCDKNTGDYYEDSYEDISAYLLSKNNAIEPRSFSQNDKTHTCPPCPAPELLGGPSVFLFPPKPKDTLMISRTPEVTCVVVDVSHEDPEVKFNWYVDGVEVHNAKTKPREEQYNSTYRVVSVLTVLHQDWLNGKEYKCKVSNKALPAPIEKTISKAKGQPREPQVYTLPPSRDELTKNQVSLTCLVKGFYPSDIAVEWESNGQPENNYKTTPPVLDSDGSFFLYSKLTVDKSRWQQGNVFSCSVMHEALHNHYTQKSLSLSPGK

SEQ ID NO: 11 - DNA, 2793 bp, synthetic construct
  misc_feature 1..2793: note = Light Chain (LC)-Fc
  regulatory 1..60: note = Signal; regulatory_class = other
  regulatory 2113..2793: note = misc_signal - Fc region; regulatory_class = other
  source 1..2793: mol_type = other DNA
atggagacagacacactcctgctatgggtactgctgctctgggttccaggttccactggtgaaataactcgtactactcttcagtcagatcaagaggaaattgactatgatgataccatatcagttgaaatgaagaaggaagattttgacatttatgatgaggatgaaaatcagagcccccgcagctttcaaaagaaaacacgacactattttattgctgcagtggagaggctctgggattatgggatgagtagctccccacatgttctaagaaacagggctcagagtggcagtgtccctcagttcaagaaagttgttttccaggaatttactgatggctcctttactcagcccttataccgtggagaactaaatgaacatttgggactcctggggccatatataagagcagaagttgaagataatatcatggtaactttcagaaatcaggcctctcgtccctattccttctattctagccttatttcttatgaggaagatcagaggcaaggagcagaacctagaaaaaactttgtcaagcctaatgaaaccaaaacttacttttggaaagtgcaacatcatatggcacccactaaagatgagtttgactgcaaagcctgggcttatttctctgatgttgacctggaaaaagatgtgcactcaggcctgattggaccccttctggtctgccacactaacacactgaaccctgctcatgggagacaagtgacagtacaggaatttgctctgtttttcaccatctttgatgagaccaaaagctggtacttcactgaaaatatggaaagaaactgcagggctccctgcaatatccagatggaagatcccacttttaaagagaattatcgcttccatgcaatcaatggctacataatggatacactacctggcttagtaatggctcaggatcaaaggattcgatggtatctgctcagcatgggcagcaatgaaaacatccattctattcatttcagtggacatgtgttcactgtacgaaaaaaagaggagtataaaatggcactgtacaatctctatccaggtgtttttgagacagtggaaatgttaccatccaaagctggaatttggcgggtggaatgccttattggcgagcatctacatgctgggatgagcacactttttctggtgtacagcaataagtgtcagactcccctgggaatggcttctggacacattagagattttcagattacagcttcaggacaatatggacagtgggccccaaagctggccagacttcattattccggatcaatcaatgcctggagcaccaaggagcccttttcttggatcaaggtggatctgttggcaccaatgattattcacggcatcaagacccagggtgcccgtcagaagttctccagcctctacatctctcagtttatcatcatgtatagtcttgatgggaagaagtggcagacttatcgaggaaattccactggaaccttaatggtcttctttggcaatgtggattcatctgggataaaacacaatatttttaaccctccaattattgctcgatacatccgtttgcacccaactcattatagcattcgcagcactcttcgcatggagttgatgggctgtgatttaaatagttgcagcatgccattgggaatggagagtaaagcaatatcagatgcacagattactgcttcatcctactttaccaatatgtttgccacctggtctccttcaaaagctcgacttcacctccaagggaggagtaatgcctggagacctcaggtgaataatccaaaagagtggctgcaagtggacttccagaagacaatgaaagtcacaggagtaactactcagggagtaaaatctctgcttaccagcatgtatgtgaaggagttcctcatctccagcagtcaagatggccatcagtggactctcttttttcagaatggcaaagtaaaggtttttcagggaaatcaagactccttcacacctgtggtgaactctctagacccaccgttactgactcgctaccttcgaattcacccccagagttgggtgcaccagattgccctgaggatggaggttctgggctgcgaggcacaggacctctacgacaaaactcacacatgcccaccgtgcccagctccagaactcctgggcggaccgtcagtcttcctcttccccccaaaacccaaggacaccctcatgatctcccggacccctgaggtcacatgcgtggtggtggacgtgagccacgaagaccctgaggtcaagttcaactggtacgtggacggcgtggaggtgcataatgccaagacaaagccgcgggaggagcagtacaacagcacgtaccgtgtggtcagcgtcctcaccgtcctgcaccaggactggctgaatggcaaggagtacaagtgcaaggtctccaacaaagccctcccagcccccatcgagaaaaccatctccaaagccaaagggcagccccgagaaccacaggtgtacaccctgcccccatcccgggatgagctgaccaagaaccaggtcagcctgacctgcctggtcaaaggcttctatcccagcgacatcgccgtggagtgggagagcaatgggcagccggagaacaactacaagaccacgcctcccgtgttggactccgacggctccttcttcctctacagcaagctcaccgtggacaagagcaggtggcagcaggggaacgtcttctcatgctccgtgatgcatgaggctctgcacaaccactacacgcagaagagcctctccctgtctccgggtaaa

SEQ ID NO: 12 - protein, 931 aa, synthetic construct
  REGION 1..931: note = LC-Fc6His
  REGION 1..20: note = MISC_FEATURE - Signal
  REGION 705..931: note = MISC_FEATURE - Fc region
METDTLLLWVLLLWVPGSTGEITRTTLQSDQEEIDYDDTISVEMKKEDFDIYDEDENQSPRSFQKKTRHYFIAAVERLWDYGMSSSPHVLRNRAQSGSVPQFKKVVFQEFTDGSFTQPLYRGELNEHLGLLGPYIRAEVEDNIMVTFRNQASRPYSFYSSLISYEEDQRQGAEPRKNFVKPNETKTYFWKVQHHMAPTKDEFDCKAWAYFSDVDLEKDVHSGLIGPLLVCHTNTLNPAHGRQVTVQEFALFFTIFDETKSWYFTENMERNCRAPCNIQMEDPTFKENYRFHAINGYIMDTLPGLVMAQDQRIRWYLLSMGSNENIHSIHFSGHVFTVRKKEEYKMALYNLYPGVFETVEMLPSKAGIWRVECLIGEHLHAGMSTLFLVYSNKCQTPLGMASGHIRDFQITASGQYGQWAPKLARLHYSGSINAWSTKEPFSWIKVDLLAPMIIHGIKTQGARQKFSSLYISQFIIMYSLDGKKWQTYRGNSTGTLMVFFGNVDSSGIKHNIFNPPIIARYIRLHPTHYSIRSTLRMELMGCDLNSCSMPLGMESKAISDAQITASSYFTNMFATWSPSKARLHLQGRSNAWRPQVNNPKEWLQVDFQKTMKVTGVTTQGVKSLLTSMYVKEFLISSSQDGHQWTLFFQNGKVKVFQGNQDSFTPVVNSLDPPLLTRYLRIHPQSWVHQIALRMEVLGCEAQDLYDKTHTCPPCPAPELLGGPSVFLFPPKPKDTLMISRTPEVTCVVVDVSHEDPEVKFNWYVDGVEVHNAKTKPREEQYNSTYRVVSVLTVLHQDWLNGKEYKCKVSNKALPAPIEKTISKAKGQPREPQVYTLPPSRDELTKNQVSLTCLVKGFYPSDIAVEWESNGQPENNYKTTPPVLDSDGSFFLYSKLTVDKSRWQQGNVFSCSVMHEALHNHYTQKSLSLSPGK